European Patent Application EP 4 600 269 A1, published August 13, 2025. Title: A Method for Preparing Biosynthetic Human Structural Material Type IV Collagen. Applicant: SHANXI JINBO BIO-PHARMACEUTICAL CO., LTD. Application WO, filed December 21, 2023. The sequence listing filed with the application follows.

SEQUENCE LISTING (38 sequences)

SEQ ID NO: 1 - protein, 30 aa, synthetic construct
GAKGDKGSKGEVGFPGLAGSPGIPGSKGEQ

SEQ ID NO: 2 - protein, 300 aa, synthetic construct
GAKGDKGSKGEVGFPGLAGSPGIPGSKGEQGAKGDKGSKGEVGFPGLAGSPGIPGSKGEQGAKGDKGSKGEVGFPGLAGSPGIPGSKGEQGAKGDKGSKGEVGFPGLAGSPGIPGSKGEQGAKGDKGSKGEVGFPGLAGSPGIPGSKGEQGAKGDKGSKGEVGFPGLAGSPGIPGSKGEQGAKGDKGSKGEVGFPGLAGSPGIPGSKGEQGAKGDKGSKGEVGFPGLAGSPGIPGSKGEQGAKGDKGSKGEVGFPGLAGSPGIPGSKGEQGAKGDKGSKGEVGFPGLAGSPGIPGSKGEQ

SEQ ID NO: 3 - DNA, 900 bp, synthetic construct
  source 1..900: mol_type = other DNA
ggggctaaaggagacaagggcagcaagggcgaagtcggtttcccaggtctggctggtagcccgggcatcccgggttcaaagggtgaacaaggtgctaaaggcgacaaaggcagcaagggtgaggttggtttcccgggtctggcgggttctccaggcatcccgggtagcaaaggagaacaaggtgcgaaaggcgataaaggctccaagggtgaagtgggcttcccgggtttagccggtagcccaggtattccgggtagcaaaggcgaacagggtgcgaaaggcgacaaagggagtaagggcgaggtgggttttccgggtttggctggctcgccgggtattccgggttcaaagggcgaacagggcgcgaaaggtgataaaggcagcaaaggcgaggttggcttcccgggtctggcaggtagcccgggtatcccgggtagcaagggtgagcagggtgccaaaggcgacaaaggtagcaagggggaagtgggttttccgggactggcaggtagcccgggtatcccgggttctaagggcgagcagggtgcgaaaggtgacaaaggtagcaagggcgaggttggctttccgggcttggcgggtagcccgggcattccgggctccaagggtgaacaaggtgcgaaaggtgataaaggctctaagggtgaggttggttttccgggtctggcgggttccccgggcattccgggctcgaagggcgagcaaggtgctaaaggtgataagggctccaagggcgaggtgggtttcccgggcctggcaggctctccgggcatcccgggttcgaagggcgaacagggtgcgaaaggcgataaaggttccaagggcgaagtcggattccctggcctcgccggtagcccgggcatccctggctccaagggcgagcag

SEQ ID NO: 4 - protein, 39 aa, synthetic construct
GAKGDKGSKGEVGFPGLAGSPGIPGSKGEQGFMGPPGPQ

SEQ ID NO: 5 - protein, 312 aa, synthetic construct
GAKGDKGSKGEVGFPGLAGSPGIPGSKGEQGFMGPPGPQGAKGDKGSKGEVGFPGLAGSPGIPGSKGEQGFMGPPGPQGAKGDKGSKGEVGFPGLAGSPGIPGSKGEQGFMGPPGPQGAKGDKGSKGEVGFPGLAGSPGIPGSKGEQGFMGPPGPQGAKGDKGSKGEVGFPGLAGSPGIPGSKGEQGFMGPPGPQGAKGDKGSKGEVGFPGLAGSPGIPGSKGEQGFMGPPGPQGAKGDKGSKGEVGFPGLAGSPGIPGSKGEQGFMGPPGPQGAKGDKGSKGEVGFPGLAGSPGIPGSKGEQGFMGPPGPQ

SEQ ID NO: 6 - DNA, 936 bp, synthetic construct
  source 1..936: mol_type = other DNA
ggagctaaaggggacaaaggctccaaaggcgaagtcggtttcccgggcctggcgggtagcccgggtatcccgggtagcaagggtgagcaggggttcatgggtccaccgggcccacagggtgccaaaggtgataaaggttctaagggcgaggtgggtttcccggggctggcgggttctccgggcattccgggaagcaagggtgaacagggctttatgggtccgccaggtccgcagggtgcgaaaggtgataaaggcagcaagggagaagttggcttcccgggcctggcaggcagcccgggcattccggggtcgaagggcgaacaaggtttcatgggtccgcctggtccgcaaggtgcgaaaggtgataagggtagcaagggtgaagtgggttttccgggattagcgggttctccgggcattccgggttcaaaaggtgaacaaggctttatgggtccgcctggcccgcagggtgctaaaggcgacaagggtagcaaaggcgaggtaggtttcccgggtttggcgggcagcccgggcattccgggttccaagggcgagcagggttttatgggcccaccgggcccgcaaggcgcaaaaggtgataagggcagcaaaggcgaggtgggcttcccgggactggcaggttctccgggtatcccgggttccaagggtgagcagggtttcatgggcccaccgggtccgcagggtgcgaaaggcgacaaaggtagcaagggcgaagttggttttccgggcctggctggttcgccgggcatcccgggctccaagggcgagcaaggcttcatgggtccaccgggtccgcaaggtgccaaaggcgacaaaggtagcaagggcgaggttggttttccgggcttggctggtagccctggcatcccggggtccaagggtgaacagggctttatgggtccgccgggccctcaa

SEQ ID NO: 7 - protein, 51 aa, synthetic construct
GFPGFPGAKGDKGSKGEVGFPGLAGSPGIPGSKGEQGFMGPPGPQGQPGLP

SEQ ID NO: 8 - protein, 306 aa, synthetic construct
GFPGFPGAKGDKGSKGEVGFPGLAGSPGIPGSKGEQGFMGPPGPQGQPGLPGFPGFPGAKGDKGSKGEVGFPGLAGSPGIPGSKGEQGFMGPPGPQGQPGLPGFPGFPGAKGDKGSKGEVGFPGLAGSPGIPGSKGEQGFMGPPGPQGQPGLPGFPGFPGAKGDKGSKGEVGFPGLAGSPGIPGSKGEQGFMGPPGPQGQPGLPGFPGFPGAKGDKGSKGEVGFPGLAGSPGIPGSKGEQGFMGPPGPQGQPGLPGFPGFPGAKGDKGSKGEVGFPGLAGSPGIPGSKGEQGFMGPPGPQGQPGLP

SEQ ID NO: 9 - DNA, 918 bp, synthetic construct
  source 1..918: mol_type = other DNA
ggatttcccgggttcccgggtgccaaaggggataaaggttcaaagggcgaagtgggtttcccgggtttggctggtagcccgggtatcccgggtagcaaaggcgaacagggctttatgggtccgccaggaccgcagggtcaaccgggactgccgggttttccgggcttcccgggtgcgaaaggcgataaaggttccaagggtgaagttggttttccgggtcttgcaggcagcccgggtattccgggttccaagggtgaacagggtttcatgggtccaccgggcccacaaggtcagccgggtctgcctggtttcccgggcttcccgggtgccaaaggcgacaaaggtagcaagggcgaagttggctttccgggtctggcgggttcgccgggcattccgggctcgaagggcgagcagggtttcatgggcccaccgggtccgcagggtcagcctggcctgccgggattcccaggttttccgggagcgaaaggcgacaagggtagtaagggtgaggtcggttttccaggcttggcgggctctcccggtatcccgggctctaagggcgagcaaggctttatgggtccaccgggtccgcaaggtcaacctggattaccgggattcccaggctttccgggcgcgaaaggcgataaaggcagcaagggtgaggtgggcttcccgggcctcgcgggtagcccgggcatcccgggtagcaagggtgagcagggcttcatgggtcctccgggtccgcagggccaaccgggcctgccgggattcccgggtttcccgggcgctaaaggcgacaaaggcagcaagggtgaggttggttttccgggtctggcaggtagcccgggcattccgggctccaagggcgaacagggttttatgggtccaccgggccctcaaggtcagccgggcctgccg

SEQ ID NO: 10 - protein, 45 aa, synthetic construct
GFPGFPGAKGDKGSKGEVGFPGLAGSPGIPGSKGEQGFMGPPGPQ

SEQ ID NO: 11 - protein, 360 aa, synthetic construct
GFPGFPGAKGDKGSKGEVGFPGLAGSPGIPGSKGEQGFMGPPGPQGFPGFPGAKGDKGSKGEVGFPGLAGSPGIPGSKGEQGFMGPPGPQGFPGFPGAKGDKGSKGEVGFPGLAGSPGIPGSKGEQGFMGPPGPQGFPGFPGAKGDKGSKGEVGFPGLAGSPGIPGSKGEQGFMGPPGPQGFPGFPGAKGDKGSKGEVGFPGLAGSPGIPGSKGEQGFMGPPGPQGFPGFPGAKGDKGSKGEVGFPGLAGSPGIPGSKGEQGFMGPPGPQGFPGFPGAKGDKGSKGEVGFPGLAGSPGIPGSKGEQGFMGPPGPQGFPGFPGAKGDKGSKGEVGFPGLAGSPGIPGSKGEQGFMGPPGPQ

SEQ ID NO: 12 - DNA, 1080 bp, synthetic construct
  source 1..1080: mol_type = other DNA
ggatttcccgggtttccgggtgcgaaaggcgacaagggttccaagggtgaagttggttttccggggctcgctggtagcccgggcatcccgggtagcaagggcgaacagggtttcatgggcccaccgggcccgcagggttttccgggtttcccgggcgcgaaaggcgacaaaggcagcaagggtgaagtgggctttccgggcctggcgggtagtccgggcatcccgggctcgaagggcgaacagggctttatgggcccaccaggcccacagggcttcccgggattcccgggtgccaaaggcgataaaggttcaaagggcgaagtcggtttcccgggtctggcaggctctccgggcatcccgggctctaagggtgaacaaggtttcatgggtccaccgggcccgcagggctttccgggttttccgggtgcgaaaggcgacaagggcagcaaaggtgaggttggctttccgggcttggcgggtagcccgggtatcccgggtagcaagggtgagcagggtttcatgggtccgcctggaccgcaaggtttcccgggtttcccgggtgcgaaaggtgataaaggtagcaagggcgaggtaggttttccgggtctggcaggctccccgggcattccgggctctaagggtgagcagggtttcatgggtccgccaggtccgcaaggtttcccgggatttccgggtgctaaaggtgataaaggttccaaaggtgaagtgggttttccaggcctggccggcagcccgggcattccgggctccaagggcgagcagggcttcatgggtccgcctggccctcaaggcttccccggcttcccgggagctaagggcgacaaaggttccaagggcgaggtgggcttcccgggcttggcgggtagcccgggcattccgggtagcaagggtgagcaaggctttatgggtccgccaggtccgcaagggttcccgggattcccgggtgcgaaaggtgataaaggctcgaagggtgaggttggttttccgggtctggcaggtagcccggggattccgggtagcaaaggcgaacaaggtttcatgggtcctccgggtccacag

SEQ ID NO: 13 - protein, 39 aa, synthetic construct
GFPGFPGAKGDKGSKGEVGFPGLAGSPGIPGSKGEQGFM

SEQ ID NO: 14 - protein, 312 aa, synthetic construct
GFPGFPGAKGDKGSKGEVGFPGLAGSPGIPGSKGEQGFMGFPGFPGAKGDKGSKGEVGFPGLAGSPGIPGSKGEQGFMGFPGFPGAKGDKGSKGEVGFPGLAGSPGIPGSKGEQGFMGFPGFPGAKGDKGSKGEVGFPGLAGSPGIPGSKGEQGFMGFPGFPGAKGDKGSKGEVGFPGLAGSPGIPGSKGEQGFMGFPGFPGAKGDKGSKGEVGFPGLAGSPGIPGSKGEQGFMGFPGFPGAKGDKGSKGEVGFPGLAGSPGIPGSKGEQGFMGFPGFPGAKGDKGSKGEVGFPGLAGSPGIPGSKGEQGFM

SEQ ID NO: 15 - DNA, 936 bp, synthetic construct
  source 1..936: mol_type = other DNA
ggatttcccgggttcccgggtgcgaaaggtgataaaggcagcaagggtgaagtcggttttccgggtctggcaggcagcccgggtatcccgggtagcaaaggcgaacagggctttatgggtttcccgggcttcccaggtgcgaagggcgataaaggttcgaaaggtgaggtaggtttcccgggtttagcaggttccccgggcattccgggcagcaagggtgaacagggtttcatgggctttccgggcttcccaggagctaaaggcgacaaaggttctaagggtgaagtgggcttcccgggtctggctggtagcccgggcatcccgggctccaagggtgagcagggtttcatgggttttccgggcttcccaggcgcgaaaggcgacaaaggcagcaagggcgaggtgggttttccgggtttggcgggtagcccgggtattccgggttcgaagggtgaacaaggtttcatgggttttccgggattcccaggcgcgaaaggcgataagggcagcaagggcgaggttggcttcccgggactggccggaagcccgggtatcccgggatctaagggcgaacaaggctttatgggtttcccgggttttcctggtgcgaaaggcgataaaggctccaagggcgaggttggttttccaggcctggctggctctccgggcattccgggtagtaagggtgagcagggttttatgggttttccgggcttcccgggtgcaaagggtgacaaaggtagcaagggtgaagttggctttccgggtctggcgggttccccgggcattccgggtagcaaaggtgagcaaggttttatgggttttccgggcttcccgggtgccaaaggcgacaaaggtagcaagggagaggtgggcttcccgggattggcgggttccccgggcatcccgggctcaaagggtgaacagggtttcatg

SEQ ID NO: 16 - protein, 36 aa, synthetic construct
GFPGFPGAKGDKGSKGEVGFPGLAGSPGIPGSKGEQ

SEQ ID NO: 17 - protein, 360 aa, synthetic construct
GFPGFPGAKGDKGSKGEVGFPGLAGSPGIPGSKGEQGFPGFPGAKGDKGSKGEVGFPGLAGSPGIPGSKGEQGFPGFPGAKGDKGSKGEVGFPGLAGSPGIPGSKGEQGFPGFPGAKGDKGSKGEVGFPGLAGSPGIPGSKGEQGFPGFPGAKGDKGSKGEVGFPGLAGSPGIPGSKGEQGFPGFPGAKGDKGSKGEVGFPGLAGSPGIPGSKGEQGFPGFPGAKGDKGSKGEVGFPGLAGSPGIPGSKGEQGFPGFPGAKGDKGSKGEVGFPGLAGSPGIPGSKGEQGFPGFPGAKGDKGSKGEVGFPGLAGSPGIPGSKGEQGFPGFPGAKGDKGSKGEVGFPGLAGSPGIPGSKGEQ

SEQ ID NO: 18 - DNA, 1080 bp, synthetic construct
  source 1..1080: mol_type = other DNA
ggatttcccgggttcccaggtgccaagggtgataaaggcagcaagggcgaggtgggcttcccgggcctggctggttcaccgggcattccgggcagtaagggtgaacagggttttccgggtttccccggcgctaaaggcgacaagggtagcaagggggaagtaggcttcccgggtttagctggctctccgggcattccgggctccaagggcgaacagggtttcccgggctttccgggagcgaaaggcgacaaaggcagcaagggcgaagttggtttcccgggtctggcaggttctccgggtatcccgggtagcaaaggcgagcagggtttccccggcttcccgggtgcgaaaggtgataaaggtagcaagggtgaggtgggtttccctggcctggccggttctccgggcatcccgggttctaagggagaacaaggttttccgggttttccgggtgcgaaaggcgacaaagggtccaagggtgaggttggttttccgggtctggcgggttcaccgggcatcccgggtagcaagggcgaacaaggctttccaggcttcccgggtgcgaaaggtgacaaaggttccaagggcgaagttggttttccgggtttggcgggtagcccgggtatcccgggttccaagggtgagcaaggttttccgggattcccgggtgccaaaggtgacaaaggttcgaagggtgaagtgggttttccaggcttggcgggtagcccgggtatcccgggttccaagggtgagcagggcttcccgggtttcccgggtgcaaaaggtgataaaggctccaaaggtgaggtgggcttccctggtctcgcgggtagcccgggcatcccgggtagcaaaggtgagcagggtttcccgggctttccaggagctaaaggggataaaggcagcaagggcgaggttggcttcccgggtctggcgggttcgccgggcattccgggcagcaaaggcgaacagggctttccgggttttccgggtgcaaagggtgataaaggtagcaagggcgaggtcggttttccgggcctggcaggtagcccaggcattccgggttcgaagggcgaacaa

SEQ ID NO: 19 - protein, 45 aa, synthetic construct
GAKGDKGSKGEVGFPGLAGSPGIPGSKGEQGFMGPPGPQGQPGLP

SEQ ID NO: 20 - protein, 360 aa, synthetic construct
GAKGDKGSKGEVGFPGLAGSPGIPGSKGEQGFMGPPGPQGQPGLPGAKGDKGSKGEVGFPGLAGSPGIPGSKGEQGFMGPPGPQGQPGLPGAKGDKGSKGEVGFPGLAGSPGIPGSKGEQGFMGPPGPQGQPGLPGAKGDKGSKGEVGFPGLAGSPGIPGSKGEQGFMGPPGPQGQPGLPGAKGDKGSKGEVGFPGLAGSPGIPGSKGEQGFMGPPGPQGQPGLPGAKGDKGSKGEVGFPGLAGSPGIPGSKGEQGFMGPPGPQGQPGLPGAKGDKGSKGEVGFPGLAGSPGIPGSKGEQGFMGPPGPQGQPGLPGAKGDKGSKGEVGFPGLAGSPGIPGSKGEQGFMGPPGPQGQPGLP

SEQ ID NO: 21 - DNA, 1080 bp, synthetic construct
  source 1..1080: mol_type = other DNA
ggggctaaaggagacaagggcagcaagggcgaggttggtttcccgggcttggcgggttctccgggtatcccgggctccaagggtgaacagggttttatgggtccgccaggtccgcagggccaacctggtctgccgggcgcgaaaggtgacaaaggtagcaagggcgaagttggttttccgggcctggccggcagcccgggcattccgggctccaaaggcgagcaaggcttcatgggtccgcctggcccacagggtcaaccgggtctgccgggcgcaaaaggcgataaaggcagcaagggcgaagtaggtttcccgggccttgctggctctccgggtattccgggtagcaagggtgaacagggttttatgggcccaccgggaccacagggtcaaccgggtctgccgggtgctaaaggtgataaaggcagcaagggcgaggttggttttccgggattggcgggttctccgggcatcccgggttccaagggcgaacaaggtttcatgggaccgcctggcccacagggtcaaccgggtctgcctggtgcaaaaggcgacaaaggtagcaaaggcgaggtcggttttccgggcctcgcgggtagcccgggaatcccgggtagtaagggcgaacagggtttcatgggtccaccgggcccacagggtcagccgggtttaccgggtgccaaaggcgataaagggtcgaagggcgaggtgggcttcccgggtctggcaggcagcccgggtattccgggctccaagggtgagcagggttttatgggtccaccgggaccgcaaggtcaaccgggtctgccgggcgctaaaggcgataagggtagcaaaggcgaggtgggcttcccgggtctggcgggtagcccgggcattccgggttccaagggtgagcagggtttcatgggtccgcctggtcctcaaggccagccggggctgcccggcgcgaaaggtgacaaaggtagcaagggcgaagtgggttttccgggtttggcgggttcaccgggcatcccgggctcgaagggtgaacagggtttcatgggtcctccgggcccgcagggacaaccgggactgccg

SEQ ID NO: 22 - protein, 33 aa, synthetic construct
GAKGDKGSKGEVGFPGLAGSPGIPGSKGEQGFM

SEQ ID NO: 23 - protein, 330 aa, synthetic construct
GAKGDKGSKGEVGFPGLAGSPGIPGSKGEQGFMGAKGDKGSKGEVGFPGLAGSPGIPGSKGEQGFMGAKGDKGSKGEVGFPGLAGSPGIPGSKGEQGFMGAKGDKGSKGEVGFPGLAGSPGIPGSKGEQGFMGAKGDKGSKGEVGFPGLAGSPGIPGSKGEQGFMGAKGDKGSKGEVGFPGLAGSPGIPGSKGEQGFMGAKGDKGSKGEVGFPGLAGSPGIPGSKGEQGFMGAKGDKGSKGEVGFPGLAGSPGIPGSKGEQGFMGAKGDKGSKGEVGFPGLAGSPGIPGSKGEQGFMGAKGDKGSKGEVGFPGLAGSPGIPGSKGEQGFM

SEQ ID NO: 24 - DNA, 990 bp, synthetic construct
  source 1..990: mol_type = other DNA
ggggctaaaggagacaaaggttcgaaaggcgaggtgggcttcccaggtctggccggttccccgggcattccgggtagcaaaggcgaacaaggtttcatgggtgctaaaggcgataaaggtagcaagggtgaggttggcttcccaggcctggctggttcgccgggcattccgggctctaagggtgaacaaggtttcatgggtgcaaaaggtgataagggtagcaagggagaagtcggttttccgggattggcgggtagcccgggtatcccgggcagcaagggcgagcagggttttatgggtgcaaagggcgacaaaggtagcaagggtgaggtgggctttccgggcctcgcgggtagccctggcatcccgggttccaaaggtgagcaaggcttcatgggtgctaaaggtgataaaggctccaaaggtgaagtgggttttccgggcctggcgggtagcccgggcattccgggaagcaagggcgaacagggttttatgggcgcgaagggtgataaaggtagtaagggcgaagttggtttcccgggcctggctggctctccgggtatcccgggctccaaaggcgagcagggtttcatgggtgcgaaaggtgacaagggtagcaagggtgaggtgggtttcccaggtttggcgggtagcccgggcattccgggtagcaagggtgaacaaggtttcatgggtgcgaaaggtgacaaaggcagcaagggcgaggttggtttcccgggtctggcgggtagcccgggcatcccgggctctaagggcgagcagggttttatgggtgccaaaggcgacaagggctcaaagggtgaagtcggttttccgggtttagccggttccccgggcatcccgggttctaagggtgaacagggcttcatgggcgcgaaaggagataaaggcagcaaaggggaagttggttttccaggcctggcaggctcgccgggtatcccgggttccaagggcgagcagggttttatg

SEQ ID NO: 25 - protein, 36 aa, synthetic construct
GLPGTPGPTGPAGQKGEPGSDGIPGSAGEKGEPGLP

SEQ ID NO: 26 - protein, 360 aa, synthetic construct
GLPGTPGPTGPAGQKGEPGSDGIPGSAGEKGEPGLPGLPGTPGPTGPAGQKGEPGSDGIPGSAGEKGEPGLPGLPGTPGPTGPAGQKGEPGSDGIPGSAGEKGEPGLPGLPGTPGPTGPAGQKGEPGSDGIPGSAGEKGEPGLPGLPGTPGPTGPAGQKGEPGSDGIPGSAGEKGEPGLPGLPGTPGPTGPAGQKGEPGSDGIPGSAGEKGEPGLPGLPGTPGPTGPAGQKGEPGSDGIPGSAGEKGEPGLPGLPGTPGPTGPAGQKGEPGSDGIPGSAGEKGEPGLPGLPGTPGPTGPAGQKGEPGSDGIPGSAGEKGEPGLPGLPGTPGPTGPAGQKGEPGSDGIPGSAGEKGEPGLP

SEQ ID NO: 27 - DNA, 1080 bp, synthetic construct
  source 1..1080: mol_type = other DNA
ggactacccgggactccgggcccaaccggcccagcaggccaaaagggtgaaccggggtccgacggcattccgggcagcgcaggtgagaaaggcgaaccgggcttgccggggttgccgggaaccccgggtccgaccggtccagctggccagaaaggtgagccaggaagcgatggcatcccgggctcggccggtgaaaaaggcgagccgggtctcccgggtctgccgggaaccccgggtccgacaggcccggctggtcagaagggcgagccgggtagcgacggcatcccgggcagcgctggtgaaaaaggtgagcccggtctgccgggcttgcccggcaccccgggaccgacgggcccagcaggccagaagggcgaaccgggttcggatggtattccgggctctgccggtgagaaaggcgagcccggcttgccaggcctgcctggcaccccgggtccgaccggtccggcgggccaaaaaggcgagccgggtagcgatggtatcccgggctcagccggtgagaagggtgagccgggcctgccgggcctgcctggtacgccgggtccgaccggtccggcgggccaaaagggtgaaccgggctccgacggcattccgggttctgcgggtgagaaaggtgaaccgggcctgccgggcctgcccggcaccccgggtcctacgggtccggctggtcagaaaggcgagccgggctccgatggcattccgggttctgcgggtgagaagggtgaaccgggcttgccaggtctgccgggcaccccgggtccgacgggtccggcgggtcagaagggtgagccgggttccgatggtatcccgggcagcgcgggagaaaaaggtgaaccgggtctgccgggtcttccgggtactccgggtccgaccggccctgcgggtcagaagggtgagccgggaagcgacggcatcccgggcagcgcgggggagaagggtgaaccgggtttacctggcctgccgggaaccccgggccctaccggtccggcgggtcaaaagggcgaaccgggcagcgacggtatcccgggtagcgcaggcgaaaaaggtgaaccgggcctgccg

SEQ ID NO: 28 - protein, 30 aa, synthetic construct
GPTGPAGQKGEPGSDGIPGSAGEKGEPGLP

SEQ ID NO: 29 - protein, 300 aa, synthetic construct
GPTGPAGQKGEPGSDGIPGSAGEKGEPGLPGPTGPAGQKGEPGSDGIPGSAGEKGEPGLPGPTGPAGQKGEPGSDGIPGSAGEKGEPGLPGPTGPAGQKGEPGSDGIPGSAGEKGEPGLPGPTGPAGQKGEPGSDGIPGSAGEKGEPGLPGPTGPAGQKGEPGSDGIPGSAGEKGEPGLPGPTGPAGQKGEPGSDGIPGSAGEKGEPGLPGPTGPAGQKGEPGSDGIPGSAGEKGEPGLPGPTGPAGQKGEPGSDGIPGSAGEKGEPGLPGPTGPAGQKGEPGSDGIPGSAGEKGEPGLP

SEQ ID NO: 30 - DNA, 900 bp, synthetic construct
  source 1..900: mol_type = other DNA
ggtcccacaggaccggcaggccagaaaggtgagccgggttccgacggcatcccgggttcggcgggtgagaaaggcgagccgggtttaccgggtccgaccggtcccgcgggtcaaaagggcgagccgggtagcgatggcattccgggttctgcgggtgaaaagggcgaaccgggcctcccgggtcctaccggtccggcgggtcagaaaggcgaaccgggcagcgatggcatcccgggcagcgcgggcgagaaaggcgaaccgggcctgccgggcccgaccggaccagctgggcaaaaaggtgaaccgggcagcgacggcatcccgggttctgcaggcgagaaaggtgaaccaggcctgccgggaccgaccggtccggcaggccagaaaggtgagcctggcagtgatggtattccgggttctgccggtgaaaaaggtgagccgggcctgccggggccaacgggcccagccggacaaaaaggtgagccgggttccgacggcatcccgggctccgccggtgaaaagggtgagccgggcctgcctggcccaacgggtccggctggccaaaagggcgagccgggtagcgacggcattccgggcagcgcgggtgagaagggtgagccgggattgccgggtccgactggtcctgcgggccagaagggtgaaccgggttccgacggcatccccggctcggcgggtgaaaagggcgaaccgggtctgcctggtccgaccggcccagcgggtcagaagggtgaaccgggtagcgatggaatcccgggtagcgctggtgaaaagggcgagccgggcctgccgggtccgaccggtccggcaggccagaagggtgaaccgggtagcgatggtattccgggtagcgcgggcgaaaaaggtgagccgggcttgccg

SEQ ID NO: 31 - protein, 33 aa, synthetic construct
GFPGFPGAKGDKGSKGEVGFPGLAGSPGIPGSK

SEQ ID NO: 32 - protein, 330 aa, synthetic construct
GFPGFPGAKGDKGSKGEVGFPGLAGSPGIPGSKGFPGFPGAKGDKGSKGEVGFPGLAGSPGIPGSKGFPGFPGAKGDKGSKGEVGFPGLAGSPGIPGSKGFPGFPGAKGDKGSKGEVGFPGLAGSPGIPGSKGFPGFPGAKGDKGSKGEVGFPGLAGSPGIPGSKGFPGFPGAKGDKGSKGEVGFPGLAGSPGIPGSKGFPGFPGAKGDKGSKGEVGFPGLAGSPGIPGSKGFPGFPGAKGDKGSKGEVGFPGLAGSPGIPGSKGFPGFPGAKGDKGSKGEVGFPGLAGSPGIPGSKGFPGFPGAKGDKGSKGEVGFPGLAGSPGIPGSK

SEQ ID NO: 33 - DNA, 990 bp, synthetic construct
  source 1..990: mol_type = other DNA
ggatttcccgggttcccaggcgcaaaaggtgataaaggcagcaagggcgaggttggttttccaggtttagctggtagcccgggtatcccgggtagcaagggcttcccgggttttccgggtgctaaaggcgacaaaggctccaagggcgaagtcggtttcccgggtttggcgggtagcccgggtatcccgggtagtaagggctttccgggattcccaggcgcgaaaggtgacaaaggtagcaagggcgaagttggcttcccgggtttggcgggttccccgggtatcccggggtccaagggcttccccggattcccgggcgcgaaaggcgataaaggtagcaagggtgaagtgggttttccgggtctcgctggcagcccgggtattccgggctccaagggctttccaggctttccgggtgcgaaaggcgataaaggtagcaagggtgaggtgggttttccgggtctggcaggtagccctggcatcccgggctcgaaggggttcccgggcttcccgggagccaagggtgataaaggttctaagggtgaggtcggttttccgggcctggccggtagccctggtatcccggggagcaagggtttcccgggttttccgggtgccaaaggcgataaaggctctaagggcgaggtgggcttccccggtctggcgggtagcccgggtattccgggttctaagggcttcccgggttttccgggtgcgaaaggtgacaagggctccaagggtgaagttggttttccgggtctggctggtagcccgggtatcccgggtagcaagggcttcccgggtttcccgggcgcgaaaggcgacaaaggttcaaagggtgaagttggttttcctggcctggcaggcagcccgggcattccgggttccaaaggttttccgggcttcccgggtgcgaaaggtgacaaaggctcgaagggtgaggtgggcttcccgggtctggcaggttctcctggcattccgggttcgaaa

SEQ ID NO: 34 - protein, 6 aa, synthetic construct
GFPGFP

SEQ ID NO: 35 - protein, 15 aa, synthetic construct
GFMGPPGPQGQPGLP

SEQ ID NO: 36 - protein, 6 aa, synthetic construct
GLPGTP

SEQ ID NO: 37 - protein, 6 aa, synthetic construct
ENLYFQ

SEQ ID NO: 38 - DNA, 18 bp, synthetic construct
  source 1..18: mol_type = other DNA
gaaaacctgtatttccag